European Patent Specification EP 3 850 097 B1, published February 11, 2026. Title: NOVEL TARGET TO TREAT A METABOLIC DISEASE IN AN INDIVIDUAL. Applicant: Universidad del País Vasco. The sequence listing filed with the application follows.

SEQUENCE LISTING (411 sequences)

SEQ ID NO: 1 - DNA, 3486 bp, Mus musculus
agcccataccaaatctctgggagactttctggctgcccatgagtaactccaggcccccaggtctccagagtgggatggtatcccgggaaccactcagagattagctaaggagctgaaggaagtccgaaaggcacttccggtccgagaggctaaacagccttcctaatctcacttagaccacagacttgccacttgagacatcagagctgaaggctgaaattcctcaaggagtcacctgggagcaagctgcgaccagcctggagtgacacatctgtattccatccgctatctccctctttgcccatccttaccctgtcctcatatgctcataggcacttaggcagaagtcatctcctcgggattctgccaaagatctgcctgttgggtttgtagggggaggataagaaaagaaagaaaagaaaaagctctgaagttgtcactttggagaagtgaagtcgaaaagtgtggcacaatgaatggacctgtggatggcttgtgtgaccattctctaagtgaagagggagccttcatgttcacatcagaatctgtaggagaggggcatccagataagatctgtgaccagattagtgatgcggtgctggatgctcacctcaagcaagaccccaatgccaaggtggcctgtgagacagtgtgcaagacaggtatggtgctactgtgtggggagatcacctcagtggccatggttgattaccagcgggtggtgagagacaccatcaagcacattggctatgacgactctgccaagggctttgacttcaagacttgcaatgtgctagtggctctggagcaacagtccccagatattgcccaatgtgtccacctagacagaaatgaagaggatgttggtgcaggagatcagggtctgatgtttggctatgctactgatgagaccgaggaatgcatgccccttaccatcgtgctcgctcacaaactcaacacccggatagcagatctgaggcgctctggtgtccttccctggctgagacctgattctaagactcaggtaacagttcagtacatgcaggataatggtgcagtcatccctgtgcgcatccacaccatcgtcatctctgtgcaacacaatgaagacatcacactggaggccatgcaagaggccctgaaagagcaggtgatcaaagctgtggtgccagccaagtacctggatgaagatactgtttaccacctgcagccaagtgggcggtttgttattggaggcccccagggggatgcaggtgtcacgggccgcaagattattgtggacacatacggaggctggggtgcccatggtggtggtgccttctctggaaaggactacaccaaggtggaccgctcagcagcttatgctgcccgctgggtggccaagtccctggtaaaggctgggctctgccggagagtgcttgttcaggtgtcctatgccattggtgtggcagaacctctgtccatttccatcttcacctacgggacctccaataagactgagcgggagctgctagaggtggtgaacaagaactttgaccttcggcctggtgttattgtcagggacttggatctgaaaaaacccatctaccagaagactgcgtgctacggccatttcgggagaagcgagtttccctgggaggtccccaagaagcttgtgttttagagccgctggaaagtttagctctgtcccatactcacctcttcaggatctcaactccctggtctcctagcctctcccagagtgccctccttgccttctaccctcagggcaaagccagcttcttctaattttcccctatccagcaatctgcaaacatcttatgaatgacatgacaggtggctttctggtgctaggttatcatgtctccttttgagggtagtcactgttccctgcctgtccctcagatgacagcaatgctaattttgtgtaaaagttactcctgtttgacaggaagtccttccctcacttcctcccatagtctgaaccttaccaggccatctcttcctccattctagatatgtacccagatgaatatattgcacagacctctggcttcccctttacatctgcagccagagattccgagccattgctatctaagggtccctctgagactaggcatctgctacataaaatatggtcaatgtctcctgagcatttgcatcgtgtgagggactgagctgtgtgttcttcatctcagcacaataaggtgttgtctttattattatccacagtaactgatggaaaactgaggctcagagagtctatgaagctctgacaagtttccatagccacatgtatcagagccaagaaatggatctaggagttctgactctaaccctcacatttgtatcccagacaagatgttgaccagagtgatgacaagtggatcgacttgaggctatggctacttatttaaggcctgggtctcctgagaattaggagatgaacctagtggctctttgtgagccctggacagcgttccacaaaatcaaaatggagacatataagtgtctcatttgttctggaagagggtttaaggaaatctgggtatcttggcctatcaagctgggctggagtctcgaactaagaggaagtttcatggtcctggcccccaacactgaaagataggtgtgtgagttctctgggcatgggttctaatcatagacagccacatgtgcttccctcctcacagaggagaggcagctggttgttatagcacagacaaccggcctctgaaaggggaccctgcaccttttgaggctttctcctttcctggacgctcatgcttatgcaggctaagtgttccaggtagagggacagcctccaagcaatcgacaagttgccaagatctcatgagaactggcttttaccaggtagcctttgaaagacatgtctgtccagcagggttctgggaaccacatgtttctaagtgtcccatcataatcagtaccacattcccaacctgtccctagttgggcccttctcacagcatactgccttcatagctcccaagaacatgggttcaggaggggacctggctcagagaaggttctggctaggagaagggctgggcagcttcatcaagaagcagataccttgcatctgtgccttgactgggcagagatcccagctttcccctttcccccagcgtgaggaaacagcagagggaaaagcctcattggccaacagatcctgatgctgtgtgtgacttagaagcttgagtctttccatagggttcggagctgcctgggagccaagttcctcacagcagaaggaaggatgggcgtgcgaaggttgagttcctgtaacttaagctttatcaaaataaaaatccagaatggtatacttgctctaaccctgagagtaatgagcctctttctttcctttcaacatttcctaggaaagaaagccattatttgttaatgttacctgatgatagtatggtgaataaaatctcaaggagcaacaacactgtacttgca

SEQ ID NO: 2 - DNA, 25000 bp, Mus musculus
aaatagtttttactgctcctcttgagttcactgtcatctatctattttaacatcacctttagttctaaaatgtactaacctgagtatctttttcctttatttttttggctgtttgtcttatttaactttacaaagaattagctattccatctaccatgcctatttatattatttgctttatctcaatttcattaatttccttcttgatctttattatttatttacatgtctaaatttcaactttggcttgttttctaagaccctgcggtacatcattaggggatttatttgagagcagccttatcttattatataaagtactcataaacttctttttgagaactgtaaacaaaaagtttcttcacagactcagcagtcaattggtttttccgagcagaagttgctacatggaaatgaggtcaaatatgagcctttgctatgttgaacttaggttatcagtagtattaggaagggacatgaggacagttcatgcgtcagggagcccaggacagcctgtgcacaagaaatattcaatttacatttagttggcaatttagagctatgatgtcttcatgggtttgactcttagaatcattatacctctgccaaggtctgttagaaaaagactgaagctactattttacatcttgtgaagatgggtgttttacataaccaataacatttattatggatgctaaacctttacctgcttcagcactgctaaatcctgcctttgtttttttggaaacatcattttgctatgaatccaaaactggcctttaaccccaaatcctcttgcctcagccttccaaatgtttcagtttacaggtgaaaacagccaatctatttccattttatatttcaccaaaacatgcttatgacaagtatatttgtgacattaaaataaatggaaaagtaaaaatattcaagcaccagggaatgagcagctgaataatatacagtacatttcttctgtgggatactgtttaggtgctaaaagaaatatctatctgtatgtcaaatatgaaaagtgagctacatatagatatgggaaaggagcaaactgcaaatatgtgtatgtgaataaacatatgcacatataccatgctctatttttgttcagaagaatagcatgcatacatgcatagcttgtttaattatatttgctaatgttcataacttcgtattgctttctagaagtatgttaaagactcattatgcctaaatagtctaatctcatttttacagtaattctataaggcaggtaataatttttcctgttgctgagctatgcaggtttgctctgggctgtgtagtagtttagagaaacaactgaggcttcagccctgaagcctgaactgctacctgcaatagtctgtgatttcttatcatttattttaagaaaaaaacaggaggtatccttgtatatagaagccatattgtccagagctcaggcaggagctagactgaatcagttgccttcaggatttttccctcactttgaattgatggcaccaatttctgaaagccctatttctgtataaagaacatctaacaggtaccctctgccccatgatgttattactcattttgaaattcaaaagagaggtgccttgttttctgtctccttgctggatctaagaaccttaaagaattattaataattagactttaagttgctcttgaagcatatttataatgttgctacagttctactagctagggtaacctaggcctatgcttcaaattacacattagtttgtattgtctctaggtttgaaactaatgtacccaaaagtaatttacaaagagacaatgatgttgaaatattttcagcacaaacactgaggcatataaagtttgcaagaccaaggggcctctcttcccaatgatggctgactaggccatcttctgcagctagagacacaagctccggggggtggggtagggtactggttagttcatattgttgttctacttattgggttgcagacccctttagctccttggttactttctctagctcctccattgggggccctgtgttccatccaatagctcactgtgagcccagtgtccctttcgatcccatgttttagcagtcatgtacctaagcaagttagctcacttcttgttaagtgctttgatagctgtgcagttacaagcagcctcgtagcatcccatatcgatttattgtagttttaatttcctagagtgactgttttgattaactaacctcaaggtttggagcactagaatttgtgccagaaaaaaaccccaaaagtgtataaagtgcctgtataagtgcagggcaggttttagccactaaggttagttgttttggacattacctcctcctattttgagcttcctccagtccactctgtaggcacaaggctttggttggttactttttattgtattctagaaggaactggtttcttactaatctcctgtctggtctcaacttcccattactcaaacattgtagatctgagagtaggagaaaacctgcagacagacgctatcatttttgacacaagctaattaaggatactatcaatcctgcatagaatgaagttataggaacttcatgtgtttatgagaggaacaaaactgaactcacggaagtttgtcacatgttggggggggggatactaaaccggaatactaatttgcacataatgaatctgtttctcaaaattccattttaaaaaattaataatctttgtgtcctggatcacccaccagcgccactaccaaacctctagcttgttaatgtgtttgcaggtctcttagagatattgacagcttaggtgatttcttgtgtcaggaaaaaaaaatgcgggcggcaaagatttccctcgaactaaagcgaatctgttgtgtaatggtacagctggttcagggtacaggtgcactctcttggctcctgttctgcgctgaggaggtagagggggcgagcccaatccagagcaggtgtgggggtggagagaagccttcacagcagagcctcactgtgttgcaaccttagcccataccaaatctctgggagactttctggctgcccatgagtaactccaggcccccaggtctccagagtgggatggtatcccgggaaccactcagagattagctaaggagctgaaggaagtccgaaaggcacttccggtccgagaggctaaacagccttcctaatctcacttagaccacagacttgccacttgagacatcagagctgaaggctgaaattcctcaaggtaaaaagacctccccccttccaggaaatggactcctccactgtccttgcttgattattcaggcactttcacttttccatatataggagtcacctgggagcaagctgcgaccagcctggagtgacacatctgtattccatccgctatctccctctttgcccatccttaccctgtcctcatatgctcataggcacttaggcagaagtcatctcctcgggattctgccaaagatctgcctgttgggtttgtagggggaggataagaaaagaaagaaaagaaaaagctctgaagttgtcactttggagaagtgaagtcgaaaagtgtggcacaatgaatggacctgtggatggcttgtgtgaccattctctaagtgaagagggagccttcatgttcacatcagaatctgtaggagaggggcatccaggtaagtaggttgccttgaactcaggtaatcctgccatccccagcctgtgccaggagttacttttactaggtaccttaaaaacaaggttcatccattgctgtagagactctttgcaggaagtgtgctttctttgctggttgtaaaggtgtcacccatcttgaagactaggaggatggttctcaaataggaaaaagttttgcatgtgagccatgcacaggttagaaaggaatagcactgcactctaatggctgctgagtcggagctgcagatggcaaggatctcagagatgcttttctgacacagtatgaacttcctaaagagcagtgcttttcaatgtgtgggtcttgactccttgagagtcaaataaccccttctcaggggtcacctaagaccaccagaaaacactgttttgaattgttcataacagtagcaaaatgacagttatgaagtagcatcaaaaataactttggttgggggttactacaacatgaggaactgtattaaaaggtcacagtattaggaagcttcagaaccactgctatagaggaacattcaaacattgttttggttcttgaaagggggatggattgtgatggaaagctacagacaattgtcagtgacaggaccctgagtaggtagtcacaagttctgactgtaggacagaggttgtcaagctgtatagtacagaggcatcacatcacaaggctcaatgacgccaagggctgggacttactcccatcgtgtccaatttggtaggtcttgataggtagatgcttaagaattctaatttataacagcttttaggaggtgctgcttctgctggtatgggaataccacattgagaacaactgatctaggagagctctggggttgataaccattgttctaggagaaacctggatttaggcacactgatttgaggatttgagaacttattcacatccttctgggcgatatgttgtgtcaccaagtgacttgtcaccaagtctaattttcctaccttccttctctctccaagagattaactttataccttgaaattcgactttgtgtttttcaattcactacacctgtgtgccttattccatggtccccaactgaaggcaatccaggccctcttctttcagaagcattttgttatgtctaggaccattttttttttttttattgttgcatcatagggcttggaggcaagattttcctggagtctgttggctaggaaccagacatgcagctaaacattccacaatacttgagtgagtcccataaccaagaattatttggccccaaatgtcaatagtgcagctgtccatcataggtacatctctggtgtttgtctgggcagctccattgtttctgatagtcacccatatgttagaagaacatactatgccaagagaaagtgaagtcttttcagtggttacttgtctcaagtgtagcccgttgtacctaacagccatgtgtttggtggacagagcaggaagacatctgctaacccactgactattttgcttcgttaatgatagcctatcaatttgtctcattcaccattcactttctactgtaaattaagtgtccaagttggttggtttccttggaggcttggtgacctgtttaccatttcatggcaaaattctcccgtactagaaagataaaatgactgtcttaagcctatgaagtaatagaaactttgaaatcctgagcagacttctcagaaagaaattcttccagggattgatgtagctcagcagtacagatagagtttgcctgccagcctatgcaagtccttgtatttagtggcttcactcctggatgggaaaaaaaaaaagatttgaattgtaatcacagcacttggaagctggagacaggggagttaagacatcaagattacccttgactgtagagcaagctcaaggcaaacttcattgtgtgaatctcaaaaatcccagatgggagggggagcgaggagagagagcaaggtctcttagggattgaggaattatcaagcatctatcttcatgaccttgctaatttttccctttacctgtatttcccaacatagtggcaccttatgtgagctggacatagtaatagtagtaataataataataataataataataataataataaataataataattcctttacatgaatgggatttctggatatctgtcagtagttaacttatgaatagcttatagacactctgacaggtcaatattgaccaccatataacttattttagaatgtcaggcggcctttactgatatgactggcagaggatgtggactcacaccttcccagatttaaaatgagcatctaccactggcagaaggatggatagaaaaactccatcatttatttcaaattagagagttgacatttaatggcaagttaatcaatatcttaatatctatatttgatagctaaactccttgactcaggatctgaatgctcagagatgatctccatgggccatagagatgctcagtgttaagggcactcactgcttttgcagaagacgggtttgatttgagcatccactccagctccagaggaccaacatctgcttctagatcccatggttatctgttcccacatgtctgcattctcccatacagattacacatgcacatatacacaagtaaaaagaaatcataaaaaaacactcttaaagaggagactctctggacattttaaacattaagtgaaagacaatatttcttaaataggaggctcttttatctcttaatttgttagtagtgtttaacggcaacgctgagtgaatttgtgcacaatgtaacttggtgatctacatgttagaaccttacttcccggctcttgctgcatctttgtcagtctcatcttagcccagctttcaggacacacgtctgacttgcaggagctgaatgaacagagggaggatctgagagcttcttatggtagtgttctcatgaacagtggtgtctatgggttctcttgtggagggaaccatggttgatgccatctacctgggtttgtgttttgtaccttttagtttgcatctatagagccttcaatatggcatttgtctggtcacttagtgaccagattttactgattttatgaaggatgttagactatagccataatttttctgaatgttagcactagggaatagggttgggaaatgaaagacttctttagtataatgtgattgtgagttgcttggactcttagaagagctggctttgaaatgtattttccttttaagggattctatgagttcatgcaatacctgccatccaaaatgagggaagaattagaagaaattaagaattcaaatactcatgcaggcaactccagtcaaactcagtggctcacctaaacaaagcagcaaaatagaggggggacctaaagaaaaagctcaaaaggaatggagggaaataagagagggtaatggggattggttatgagcaacatatattgtacatatatacatatgtatatgcatatatatatacatatatatatgaaactgtcaaagaatagggaaaattaaaaatctataaaaggatttattagacaaaacaattctcatttttgatatgtaagagaatatcctttttatttttgatagataggtttgataagctgactcataaggtgtcttttttagaatttaagtttgccatgcttagcaattatgttacttgttacattcagtgtttgttcttatccagataagatctgtgaccagattagtgatgcggtgctggatgctcacctcaagcaagaccccaatgccaaggtggcctgtggtaagagacaagttcccttttttttttttttgctggagacctaagtatgctggacaaagaagttcatggtgcacatagatcatagagtcatattcaagtccaaagtcaatgtcctcctgtctacaggagaggtcttcttaaagtgactttcttatgttgtataagggcagaaaacatttctaatgatgaaacagattcatcacctagaagttgatgtaagatgtcaccagaactagcagaggactaggggggaacatggtctccttagcaaaggtttcactgggagtcggtggactttctaaattcttagatgaatccttccgagaaagtgaagagctgaaatgcttgaggctggctagaaactcagttgatgactatgtatatctagctactttgattttctttccttgtttgtggtatgcctcatatgttaaattaatttatgcatcccatttaccagcaacaaagaacagcagtttcattaactattcacacccaaaccaacagcttttcaaagggccatcagtgttgaataaagcactgaagcccttgtccacccatgccatccacctgtggtctctgggggtccatataggccaaatatctttactgttgtttgcaagataagttttccagcatcaaatctttgtctgatagaaggctttgtcacacaacatagtccttgacttcagagtgtggaaggtccatgtccaatctctgaccttacagatgggaagacagtgctggttgcacctggctctttgccataccttatggtgcaggagaccccagtgtggagaccagtatgcactgtcactgtctgtgatgtatactgtcctctgtgaagaccctcccttccttctctacaagcatctcagcccgtatgtcaggtccttgttttactctgagagtagatatcaccctgatagcattgaaacaaacagtggcattttctgtaagattttggcattgtatccacactagattcttagctagggctcttgctcctgtttttaaagattccatgagagcctctggcagtagatagttatgggattccagttcttacagaaaaattccttttgagaaagtggtctgatttgatccttgggttaggatacacatgttctagcatcatggtctctgtgtatgtgtgtatgtgtgtgtgtgtgtgtgtgtgtgtgtgtgtgtgtgtgtgtgttgagagatgttgtgtcatatgcattcatcctgttgattaattcatgaaagctacatgactggagacaggttaagtaggttgtccaagataacagaatcagtaagtactttgcacaaaactcaaatacaactcatccttttcaaagcttcattctactaccaacacttgcacatactcagtaattagtgctggagttgctctttttgttggcacagctattctttcttagaaactattcttcactgaagccactaatgaatcgttctatctccactttgataggtctagacacttgagcttctgtcagctgcccatgactactacctaccttccttttcttacagagacagtgtgcaagacaggtatggtgctactgtgtggggagatcacctcagtggccatggttgattaccagcgggtggtgagagacaccatcaagcacattggctatgacgactctgccaagggtgaggatgagtttgctgggtctgtgtgcatgtaggtctctgctgtgtccattttccatacggagtcaaatctgatccttcagttttacagtacaaattccatctggagagtaaacattcctagagcaaggtctggctgccttctatagaggactacagcgggaggggccagcgtgtatctgttcattactgacaagtctcttttaaggtcctgctttccctgtgctggcagaagctttgaatgaagctcgtaatgaagggggtatccctttagtgaccacaagctctgtgccaagcacaggtgctagtgtctacttatgtcatctgacttcatcattccagaataccctggactgtttcttatgcaaatgaggatatcctggcttagagtataactaccgtgaaacaacaccagggtgggtgttcctgtactttccactgagctgtactgcattttactatagatacagaaaatgaggcctcattttcaagcacctgggcctaattacaggtgaaggagactgggaagtccaggttagcacccatgccaggtggttaaggagctgagggccgggaaagaggttcaggccaggcaaggaagtaaggggaccaggaagcaccaagtggcacaaggataactgaggacttccctgcagatgccactgcttatatctgggcatggcaggaagcaaccaagcctgggggtatatcagatgacccagggcatggcacttgctgcaaagacattttggtggagcttccatttgcccattattcacaccagtttcctggaaagggctcagacctgacttcttcaaggttctactatagcttctagcaatagatattcatataatttcagtttttatttctcagatttatttatttaaaaaattccctctgagtctaggttgaactctgagcctcagtttccagagctcactgtgagagatgtgttgacctagagcaatcatgagaaagaccacttcttgcagtgtgggaatgttctagagtgcctgggaaaagaaacagtatatgcaaattaatcttcccacttaagatgtgtggccttcaataagtgcttactgacagaagcctgttatagctatcttcagagaggctctacctgtgcctgacaaataaagaggtgtatcctcactgccatccattggactgagcacagtgtccccaataaaggagctagagaaaggacccaaggagctgaaagggtttgcagcctcataggaggaacaacaatatgaactaaccagtaacaccagagctcccagggactaaaccaccaatcaaagagcacatgtggtgggacttatgtctctagctgcatatgtagcagaggatggcctagttggtcatcaatgtgaggagaggcccttggtcctgtgaaggctctatgacccaatgtaggggaatgccagggccaggaagcgggagtgggtgggttggtgagcagggggacgggggagtagggggttttcggaggggaaactgggaaaggggacaacatttgaaatattaataaagtaaatatctaattaaaaaagatttgtggcctttgtagaagaaacccatcatcctgaaaaatggcgttttggaatgttaccatgcatagcctctccttggtatactctgagacttcaatttatttatgtgcatctatatcttactcaataccatgccttccattaggttacaaagaaaatttccataaggcaatgttctttagaaagggctaagtgacagcccgactatggcaaaattgaactcagcattgggaagaggtattatttcgactcaatgcttaatatacagagcagagtcctttggcacctctctaaagattattcattgatttctacatccaaaacatttactggggaatggtgggggtgagggaaaggcaaagagcaaagaaaaccacgtgcatgggtagagggactgcttggcctcatatgaccagctctgaggtgttctgtgcgaatctctttttatcttatgcaatatgggagtagaattgcatgggtaaatgtccaaggacactaactgggagctggtcaagtttgggtgttgggggaggatccagaggaggaacattccatccagagagacctcggggaggtggaaaagtgcataatgcttaaggctagacctaagtttgttgtctaaaggagttctggctccctgacaggggtggctgttagtgaggctttcttgagatatcacacagcatgcagaggtgcacctcaactctgtattgcagttttgcagatggggacttggttccagagttgtagctttgacaaaggaccccagctctaggagtctctctcgatggttcaaatacatgatacttattattcaccatgtgtgtaaataataaatatatacacacatatatacacacatatatgggtaaggtatatagttgggcctctaaatgacaagattcgaaagacccttgattttcaatcactgcagtgatattctcttctccctccttccctcccctgccatccctccatccatctccctttctctttcttttcctttctctcagacccggttcaaagtagtccagactagccaagatggcctcctgccttcacttcagaagtgctggggttacaagcaggcaccatgccttgctagtgctttgattttttcaagtggggttctggagggttctctgggatacccaccatatgttgcttacctgctcatcagtcagaatgtccttgatgctgtcaggtttgtaacgttgttgtgggttgtcacagttctgtgtaagatatacttttttttttttaaccaaggtgtaattgaatacagtaaaatatatcatggagaatcttctcttttgaaagagttctacatgatcatggaggcaaatatcaggtctttcaacatcacagtcctcacctcaactgtgaaccagaggctaccacccctaacaataaatgccacaccagtgactgagaagttcaccaagaaacttatagtcctgtcttgacacatgtccccactcggcttacttctgcccaggctttgacttcaagacttgcaatgtgctagtggctctggagcaacagtccccagatattgcccaatgtgtccacctagacagaaatgaagaggatgttggtgcaggagatcaggtatgtcagctgtgtgaggggtggaccagtgtggtgtgtttggacagagctatgatccataaggggaatcctgctgagctaattacactcttgggtggtctcatcactctagaaacctggggaagatcatgcctacagtaagttgagcactgctacccggcatcaatgtcaggatgtgtggtagaaacccatgattgctgatgacagatgtagacttgtctcctccttccagagtgttgggggtcagaggcactgtcttctccttctaaaatgctaaatgcagcagtgttttgtgtatgagagagatactgcataactgttgaagtaccaaaagaaatatgtgatttggagaatagtgctgccctgagttctaaggcagctgtccttcctcagggtctgatgtttggctatgctactgatgagaccgaggaatgcatgccccttaccatcgtgctcgctcacaaactcaacacccggatagcagatctgaggcgctctggtgtccttccctggctgagacctgattctaagactcaggtgagctgtttccatcacccccgcagacctccctactaaattataccaaatcattttggttctgggcacatttttcccaagtaatacatatttattgtcacctgccaaaatgcttttaaaatacctatattttaattcattctttgacaacacacacatccaccccacatgcttggttatatgacatgttatacacacacacacacacacaaccacacatatacatgcacacgcacacacatcccacatgcttggttacatgccctgttacacacacacacaggcacaaccccccacatactcagttatatgctgttatacacacacatacacacacacatgaacatatgcacattcaacccctcatgcttggttatatgccctgtgagccctcccttttctccctcccacttccatcaagccctccttttctctaagcagtcctccctcccccttttatgtgtttctttgtgtggataacctgctgcatttaattatagttggttgcatgaacacagctaaggggttacttatttgaataaaggtaactgactatttcttgcctacagttcctcagggagagtgggatgttatgagcctctctcctacccacaatgacacacggatgggcccaaccttgtttgcaggtagtatgcagatagccaaagcgcctgtggatttatggatgcagtgccatgttagatccagaagacaccatttcacaaccctctttcctgacttctggctctgcttgtattctttccaccctcttttccatcttgttccctgaatgttcaaaggagatgggaacattccatttaggaatagacattcaacgatcccttttcctcggcactttgatcagctgtgagtctctgtgttgtcagcacctactacaaagaggatcttctccaaccaaggtcaacacgttagcaatttggcggtataaatgtaaatatttagatggcagcttcatattgtgtctgtttagtaaagcaacaggaataggttcctcactagggcttatgctctccccagccatggggttttccatgccagatatgcatttcctcttgcggagggagcctccaatctaattagaaagtgtttgattacactttagtcatgctatttttaagatgaaaatattctacttaggtacccaaagcattatccattttgaaaggaatcacttacttgaaaactctttcaggctacacacatttcccatcctgaccctcatcaaaatttattataaaactattcaaaaaatcagacaggcttaaaaaattattctatttttattttgttagcatatgtggtctttggtggtaacttaatacctgccacagttttactacctcaccagttcctgacatggtggctcctgcctttatgagcacacagctttcccaccatgagcaggctgtatctctaggacccctttccttgtctttacccttcatgtgtcccattccagctctgtgggccttgacctccctccttcccatcatgatgaaatccctttctctttgaaggacagtggtgatgcaaacattagcacaggtggaggcaggctccctaccactcttcagtcgtctgatggcctttggccaatggctgcctgccctggctcctcttctgtgttctaaagtatgatgtcccaaggtcttgacacatcatcccctacatgttatctctatctcttcactcacttggctcctgaatcttccaaccttggtccctccacatcatcagccccatttctcactcactttacaggctcagaggccgacagcctacgctatgctgctcactatcatctcttactcggcacaggactaggtggagcacaacacattccccaggccagctttgtgccatctgtctccatggtactagtgtctcgtatttctccagaaagagtattcctctcattgcagcccaacctttcctggattggtccctacatcatccaagccagcaacagtaccctatgcccctaaaaggttctccctgcttgagaactgcagttaattttttgtgatcttctccaccttttcagaattttctctaggattttacttcttgtgagaggagggcagaattcacttgtcattccagaattcagaattgcatattattccaccataactttcctctgccagcccttttcacagagtctccaattcaccagcattaccccattcaatttatccttggttcatagggcttatacaccatcctttattgtatctgtgttttttctttggggacagcaatgcctatgtctgaatgctacttgtggcccctcataccagactgttctctctctttccccctcctcccctcttccatcccctcccttctctcccccaacccccatacttgtgattgatatagatgcttttatggcccaatatagtgcatgtagctatgtcttgttattctagtctatgtcattctactaagatgtatccttctttctgggcagaagtatcacactggctccacttggggcaactgtgtgtgcttatggtcctaatagaacattttcttagagattcctgtgcttgtgctatttttatgactttcaaggtagagttggggccaccagcatctctcaggtattgccggaggttatgggacagaagagctaacatgtagactgctgtggtaccaaaagaaagggcttagaaatgtggagttccacagaaaagacaaccccagaataggggtgagtagaagacaatgggcaccctgaagtttccttttcctctggtaagagaggaacagaaggaatgctttgagctacagtaagaaagaccttgttcatttcccctgtacaagaaagaggtttccaagtcttaggagctctgagggaaataggaagtctaatgggatgcccttttctgagaagatgcattgagtctccataagatgcagtagatatgcctgtcacagggggccaggagacactggatagttgagctgcctcctaggtctgcctctatgcagggagtactatccaggacagtagctggcctcttcctccacaggctctttgtaaaggatttccattgtcacctgtgttgactgtgaccaggatgagtctttccacctgaacaaattgctgctgctgatactgagaatcagggctggcagtccagtggctatttttgtaccaggtcagagctctgttttccatagtgtgtttttccccgtatctgctgacatgatgagataagagcagagctcgggcctttgctctgccaacccgttccaggagttctgcaaagatgcagcctggtatttgcccagtagggatgggacatcaggtctcagtgaaaaacagctagattgggaaattgcctcaagactgaacctcctcccaaggctatatgagataactttgatcctagagcctgataaaggtctcctcccttgggagtccccatccctattctacctcccccttgtgcagtcctatgagaggataattcccatggaggatttaatgggtagtcctcaatgattgtgtaccttccaatctcagatgataggtggccagagctctttttgtctctccccctggatgtctctctgttgctttttggaccagcaggacacagagcagaattccgatatgtaccccattggctatacttaatcttagctgaaagattcaaaagtgtcaggtgactttggatggctgtctaaggcaccttggccaagcagagaccatatttcagcacaacctcatcaagggactgattgctgcaaggtcctatctgggccctaggataaaaaattattctatgccacccctgcttaggtttttggtatattataggcatactgctgcaagcatctcatgaccctcagctgtgcagatactgctctgataggtacatattgtctcaggtagcatgggccctgtcatccaacagatggttcatggtcttaagtggcaactttctgctaaacagagccttggctataaatctgtgtgtcagctcttgtgtgtgatcttgaccaaaatgtttgaatgggcaacaaaggtgacccattcatgccatggcttctacctgcaaagcttgttcacccattgcatttttcttgacctcctcatctgctgacctcccaccaagccttccactttgcaaactcaaggggacctatctgcttttccttgctatctgagatatcatgtgtctgtgcccagtgatatgtcattagaggacagagtctctacagagcattttgtctgtgctacaatgagagtgacaagctttggttcagcttgagcaaggtctggatcttggactcctcacaaaatgacaagttctgatctcttggtttatgtcatttgtaaagtgtaggtggacatgacacctccctcactgtgatatcttagatcttaatctatatgatgggaaccgaactggacatgatggaagtgaatgtttgaggggtctccatggcttgccctgacaggaccttataatcaggatcctgactcctacccaagtatgctccacttgtccttcttttggtgaaacaccaagacaatggggattcagagctttctgcccttttagcttaacagtcctgactagagcctctttcacctgtccatacagctgtcaaactctcctggtcccaatgtacttccaggatcctttactgaggagagagggccacttgccaggctctttctctctgtctcagaggctctatatgccaacaaatacagtcgtggctaaagatcctttttggttcttcacattctaggaccaagatacccttgtctctgccaatgaattcctgtgttcactaatagaaatgggagaagtccatgggaagtgtccagagagggtcattagcactagcagtctcttattatcacagttgaaagacagtgccccatatgtgtgccttatgctgtcatcacagtatagagcaaattactaaatataagcatgtgccatcttcagtctccaaagaacctttagagacaaagggactctctggatcccttgggaactcaggctgcctcctggagacctgtgcctgacagccatgtgccctcagctcaggcctgggcctcacaggatctcctttgatggacaggtaacagttcagtacatgcaggataatggtgcagtcatccctgtgcgcatccacaccatcgtcatctctgtgcaacacaatgaagacatcacactggaggccatgcaagaggccctgaaagagcaggtgatcaaagctgtggtgccagccaagtacctggatgaagatactgtttaccacctgcagccaagtgggcggtttgttattggaggcccccaggtgcgtatttatctctagataaggccctgtttctgggccttgatacctggactgctcatgtcccagagtacacagatgacaagatgtagttctgaggatctcagtagtgtctgcccatgaattaaaggtgctcagtgaactttggcctacattgaagacactctgtatatctgtcaatatggaaaaaggggtacatgatcagaggagtttcccacttaatgctgtcaagccctcccacctagccattccaaatgccaccatgcctgcccatagccaccgtcatttctccctacttggtcaggcactcactcatctctgtagtgcttgttcatggctactttctcaggcattacttgctggaactttgctatgggggtctccagctattgttgcaaggacagcagaggtgagttttatagaagatacagctcttaccccattctcctatatgtacacagaccagagggggtagagattagcagaactgagggtattatcacaaggttgaacccccaaaataggtcctatggtcaaatagtgttggaataaggcagaaggttaagttccttattttcctggaggatgtctcaaagtctaaataggtaactgcaaagtgtgacttctaaatagaattgaagtaactggattctcttcaaattgctaaatctagctccatttaaaggtgtttctttcaaactgctgctaaacagagcacacttcataagtgagccacgtggtggcactggccaggatgacagcctggggttgtatttattgcagtacaattcctactacaggtggatggcttcttatggtggactcaaaagtgaaggcatggccccagatgacctctgtctcatctcctgacctttctagtaaggctttgacaggttgcctgattttcatagctggtcagtgccaggaaggacggagatgagagaactcacagtttctgcctggttcatgggggcctttgagagtgctcacaggagactctctgtcctttcttctgcccagtctgcactcagtgtcagtgcttctcatctcttgtccgtttgtctccctctgtagggggatgcaggtgtcacgggccgcaagattattgtggacacatacggaggctggggtgcccatggtggtggtgccttctctggaaaggactacaccaaggtggaccgctcagcagcttatgctgcccgctgggtggccaagtccctggtaaaggctgggctctgccggagagtgcttgttcaggtaggttgcccccacctgttgtgatccttttttcctgtgcttgccaaaggctccagcccagcctggagtaaggagatactggcccagtaggaaagcctttttgtcactgttgcatctctgcataaattgcactggcgactgtggctggagccctggcaaactagggaaagagagagcacacctgaagacagggggctgctgggcaggagaggtagggatcctattggcagaagaagtttggggcctgctgcctctgctctttaaagtctgtgagaggctcagtccctgagccagatctttcttgaaggtgtcctatgccattggtgtggcagaacctctgtccatttccatcttcacctacgggacctccaataagactgagcgggagctgctagaggtggtgaacaagaactttgaccttcggcctggtgttattgtcaggtaaaagggccatcatgttgctattgcctggaaccttcccacttccacactcaggtggacacccaaacataaagggctcttcagacacttacaacaggagggtcccaaatgcctggcccctcagcacagtgcctggaatcatagatcagtacatgcccccaacttggggtgtctggtttccagcagaaggaggcccagtggagagtagccataatgagtccatctttgagcagctggagcatctcaggccagatgtctaggaagccagtaggcaagtctattcctacatgccatcatggcatccctattctctggttcttggctgtgagagcactggccttggctaaaccagtggagtagagtagagaaagttacctcaggtaagagttcataccctggtcttggtgtgttagtactcagctgtctctgaccttggagctttcacttcttaacctgatcatgatagcactgtgttgtagatagggtacagatgtatgtgtttgtgggagaaagcctctcctaggaccacccctagtactcactaccatttcccattgaaaaatgacctttgcctcccctgactatgcagggacttggatctgaaaaaacccatctaccagaagactgcgtgctacggccatttcgggagaagcgagtttccctgggaggtccccaagaagcttgtgttttagagccgctggaaagtttagctctgtcccatactcacctcttcaggatctcaactccctggtctcctagcctctcccagagtgccctccttgccttctaccctcagggcaaagccagcttcttctaattttcccctatccagcaatctgcaaacatcttatgaatgacatgacaggtggctttctggtgctaggttatcatgtctccttttgagggtagtcactgttccctgcctgtccctcagatgacagcaatgctaattttgtgtaaaagttactcctgtttgacaggaagtccttccctcacttcctcccatagtctgaaccttaccaggccatctcttcctccattctagatatgtacccagatgaatatattgcacagacctctggcttcccctttacatctgcagccagagattccgagccattgctatctaagggtccctctgagactaggcatctgctacataaaatatggtcaatgtctcctgagcatttgcatcgtgtgagggactgagctgtgtgttcttcatctcagcacaataaggtgttgtctttattattatccacagtaactgatggaaaactgaggctcagagagtctatgaagctctgacaagtttccatagccacatgtatcagagccaagaaatggatctaggagttctgactctaaccctcacatttgtatcccagacaagatgttgaccagagtgatgacaagtggatcgacttgaggctatggctacttatttaaggcctgggtctcctgagaattaggagatgaacctagtggctctttgtgagccctggacagcgttccacaaaatcaaaatggagacatataagtgtctcatttgttctggaagagggtttaaggaaatctgggtatcttggcctatcaagctgggctggagtctcgaactaagaggaagtttcatggtcctggcccccaacactgaaagataggtgtgtgagttctctgggcatgggttctaatcatagacagccacatgtgcttccctcctcacagaggagaggcagctggttgttatagcacagacaaccggcctctgaaaggggaccctgcaccttttgaggctttctcctttcctggacgctcatgcttatgcaggctaagtgttccaggtagagggacagcctccaagcaatcgacaagttgccaagatctcatgagaactggcttttaccaggtagcctttgaaagacatgtctgtccagcagggttctgggaaccacatgtttctaagtgtcccatcataatcagtaccacattcccaacctgtccctagttgggcccttctcacagcatactgccttcatagctcccaagaacatgggttcaggaggggacctggctcagagaaggttctggctaggagaagggctgggcagcttcatcaagaagcagataccttgcatctgtgccttgactgggcagagatcccagctttcccctttcccccagcgtgaggaaacagcagagggaaaagcctcattggccaacagatcctgatgctgtgtgtgacttagaagcttgagtctttccatagggttcggagctgcctgggagccaagttcctcacagcagaaggaaggatgggcgtgcgaaggttgagttcctgtaacttaagctttatcaaaataaaaatccagaatggtatacttgctctaaccctgagagtaatgagcctctttctttcctttcaacatttcctaggaaagaaagccattatttgttaatgttacctgatgatagtatggtgaataaaatctcaaggagcaacaacactgtacttgcagtttatggtgtgtgtgtgtgtatgtccaagggagggtactgggacactgggtatcctactccattatattctgccatactcccttaagacagtctctcactcaactgagggctaggttggtggccaccaagccctagggagcctcctgtcgtcatccctgacctccactgtgctggagtgacaggggtgcacatgaccataccaagatctttcagatgagtgctaaggatttgaactcaggttttcatgcttgtacagcagtgctcttcttccctaagtgatctttgcagacctactacgcttggttttgtttgcaaaacttgagctgtttcactgtgaagcacttctgactctttcacctgcagaaaagctgggtgctattttcaggattacccaagccctgacctgtatgggacctcctcaacctctgtgagctaacacgcactgacccattcctgtactgtcagcgggttactatatccgcatcatggcctgttaaggtagagattcttactaattcttcttgtcaagtcctggagctgtgtggaagcaagtgtggagctggaactcttgaaatttcctaggaggagatattgaggcaggcatcaaatttgggacacatgcttgaagcaggctgagggcggggcaatatcacttcttagtcccatgacttgggtttcctggtgtctaactaagacccagacctattgctgggaggagaagacagagaaaacacctaatgacatctggtctcaggtcttgggtgtcgttggttctatattcagagcagccactcgttcctaatgttcctaaaggtagtaacttcacagaaaagtgaccttcaagaatatctgtgagcagcaagacccccgtgaaacatctgggaatgcttatttgcaggatggaggtttatgaatgaaaaaagggaaaaaccattactaaaaggaagaaagtgaagggctcaaaattccagcatggttaggacaggggctcatgaacgtccaccaaccaccaaagagctattggcaatggtgatgctggggacagaagagtcagtttccttcagggatacaagccctgagaggctttagtagatggtcctatatctatgcacatacatgcatactaaatggactctgggttttgttttatttttgttgttgttagtgttttgtattgtttcccatgtgaagttgggaaaaaatcgtggtggggcataggggcaaaaatgaaagggaggaaaatgggcagatttggtcaaaatgcgttacaggcatgtttgacattctcagtaaaagtagaggggaaagctaggaagttggctttacagttaaggtgcttgctgtgctagtggcaatcataaagattagaattcagatccccattatccaggttagtttcaggtgggtgtggcagctcacctattattccagcactcagaatatggaggcagaaatagccaaaaaccaggtggctagttagacaataccaacaaagtctgggctcaattgagagatcctgtcttaagaaataaggatgagagtgaatatggaagattcccaatgtcagtttccatgtgtgaggatacacatgaggacaggcatattcacatgcacaccataaacagacacacgcagaaagaaagaaagagaatatacttttgagccttggaacactcaaaggtcaagatcatagcaaaatatggatgcctttgttttctatcagtgtgataaaacaccatgaccaaaggcaacatggtaagaaaagggtttatttcagcttatagttttagtccaccataaaaggaagtcagggtagaaacctggaggaaggaactgaagtcgtggagcaacactgcttactggcttgttccttatggctggctcagccccctgtcttatacaatccaggatagcccagagtgacaccacccccatgagctggtacttcccacggcaattatttgtcaagaaaatacccaaaggcttacttataggcaatcaagaaaatacccataggcgtgtctataggcagtcagatagaatcattttcccagttgagtttccctctcccccagatgtgtcaagttgacaaaacaaaaacaaaaataaacaagcaaacaaatacaaaacaaaaaagacaacccaaatggagaaaataaaacaccccccaaacaacaacaacaacaaccaaacaagcaacaccatagaagaagcaaagcaagttgggagggcacagctagcatggaagaaggagccccagtaggtggttcatcattggaagtcaaggctatgagaactactacttaagagttcagcgcggcccaagagtgtcttacggggccaaacatctattctatgtgaggttctgtgtaactttcctgcaaatgtgttgtgaatcatcaataaatgtttttagttaaaaatattgtgaaatgaaagtatattttctctcaaattgcatcccaccacttttagaaacttatagtatctaatcaactgtgcccattaaactcatccccattacaatgttttagaacatacaaatcattagttttaactatatgacactg

SEQ ID NO: 3 - DNA, 21 bp, Artificial sequence
  Primer
gagccttcatgttcacatcag

SEQ ID NO: 4 - DNA, 20 bp, Artificial sequence
  Primer
gtcttgcacactgtctcaca

SEQ ID NO: 5 - DNA, 28 bp, Artificial sequence
  Probe
agatcttatctggatgcccctctcctac

SEQ ID NO: 6 - DNA, 20 bp, Artificial sequence
  Primer
gcactgcatcactgatctgg

SEQ ID NO: 7 - DNA, 20 bp, Artificial sequence
  Primer
tggcttgtgtgaccactctc

SEQ ID NO: 8 - DNA, 20 bp, Artificial sequence
  Synthetic oligonucleotide
agtctcccagagatttggta

SEQ ID NO: 9 - DNA, 20 bp, Artificial sequence
  Synthetic oligonucleotide
ttcggacttccttcagctcc

SEQ ID NO: 10 - DNA, 20 bp, Artificial sequence
  Synthetic oligonucleotide
gtctgtggtctaagtgagat

SEQ ID NO: 11 - DNA, 20 bp, Artificial sequence
  Synthetic oligonucleotide
caaagagggagatagcggat

SEQ ID NO: 12 - DNA, 20 bp, Artificial sequence
  Synthetic oligonucleotide
cgacttcacttctccaaagt

SEQ ID NO: 13 - DNA, 20 bp, Artificial sequence
  Synthetic oligonucleotide
gggttttttcagatccaagt

SEQ ID NO: 14 - DNA, 20 bp, Artificial sequence
  Synthetic oligonucleotide
gtcattcataagatgtttgc

SEQ ID NO: 15 - DNA, 20 bp, Artificial sequence
  Synthetic oligonucleotide
ggcctggtaaggttcagact

SEQ ID NO: 16 - DNA, 20 bp, Artificial sequence
  Synthetic oligonucleotide
tgtagcagatgcctagtctc

SEQ ID NO: 17 - DNA, 20 bp, Artificial sequence
  Synthetic oligonucleotide
gacaacaccttattgtgctg

SEQ ID NO: 18 - DNA, 20 bp, Artificial sequence
  Synthetic oligonucleotide
ccacttgtcatcactctggt

SEQ ID NO: 19 - DNA, 20 bp, Artificial sequence
  Synthetic oligonucleotide
gggctcacaaagagccacta

SEQ ID NO: 20 - DNA, 20 bp, Artificial sequence
  Synthetic oligonucleotide
tccagcccagcttgataggc

SEQ ID NO: 21 - DNA, 20 bp, Artificial sequence
  Synthetic oligonucleotide
gctataacaaccagctgcct

SEQ ID NO: 22 - DNA, 20 bp, Artificial sequence
  Synthetic oligonucleotide
agcctgcataagcatgagcg

SEQ ID NO: 23 - DNA, 20 bp, Artificial sequence
  Synthetic oligonucleotide
tggcaacttgtcgattgctt

SEQ ID NO: 24 - DNA, 20 bp, Artificial sequence
  Synthetic oligonucleotide
ggttgggaatgtggtactga

SEQ ID NO: 25 - DNA, 20 bp, Artificial sequence
  Synthetic oligonucleotide
gcccttctcctagccagaac

SEQ ID NO: 26 - DNA, 20 bp, Artificial sequence
  Synthetic oligonucleotide
gactcaagcttctaagtcac

SEQ ID NO: 27 - DNA, 20 bp, Artificial sequence
  Synthetic oligonucleotide
gcaagtataccattctggat

SEQ ID NO: 28 - DNA, 20 bp, Artificial sequence
  Synthetic oligonucleotide
gagaaccatcctcctagtct

SEQ ID NO: 29 - DNA, 20 bp, Artificial sequence
  Synthetic oligonucleotide
ccatccccctttcaagaacc

SEQ ID NO: 30 - DNA, 20 bp, Artificial sequence
  Synthetic oligonucleotide
tgtggtattcccataccagc

SEQ ID NO: 31 - DNA, 20 bp, Artificial sequence
  Synthetic oligonucleotide
gtcgaatttcaaggtataaa

SEQ ID NO: 32 - DNA, 20 bp, Artificial sequence
  Synthetic oligonucleotide
tctcttggcatagtatgttc

SEQ ID NO: 33 - DNA, 20 bp, Artificial sequence
  Synthetic oligonucleotide
ttacttcataggcttaagac

SEQ ID NO: 34 - DNA, 20 bp, Artificial sequence
  Synthetic oligonucleotide
gctattcataagttaactac

SEQ ID NO: 35 - DNA, 20 bp, Artificial sequence
  Synthetic oligonucleotide
ggcccatggagatcatctct

SEQ ID NO: 36 - DNA, 20 bp, Artificial sequence
  Synthetic oligonucleotide
tgggctaagatgagactgac

SEQ ID NO: 37 - DNA, 20 bp, Artificial sequence
  Synthetic oligonucleotide
ccaaccctattccctagtgc

SEQ ID NO: 38 - DNA, 20 bp, Artificial sequence
  Synthetic oligonucleotide
agacaccttatgagtcagct

SEQ ID NO: 39 - DNA, 20 bp, Artificial sequence
  Synthetic oligonucleotide
gttcccccctagtcctctgc

SEQ ID NO: 40 - DNA, 20 bp, Artificial sequence
  Synthetic oligonucleotide
gttgctggtaaatgggatgc

SEQ ID NO: 41 - DNA, 20 bp, Artificial sequence
  Synthetic oligonucleotide
ggacatggaccttccacact

SEQ ID NO: 42 - DNA, 20 bp, Artificial sequence
  Synthetic oligonucleotide
gccctagctaagaatctagt

SEQ ID NO: 43 - DNA, 20 bp, Artificial sequence
  Synthetic oligonucleotide
gtgcaagtgttggtagtaga

SEQ ID NO: 44 - DNA, 20 bp, Artificial sequence
  Synthetic oligonucleotide
cccccttcattacgagcttc

SEQ ID NO: 45 - DNA, 20 bp, Artificial sequence
  Synthetic oligonucleotide
gtgttgtttcacggtagtta

SEQ ID NO: 46 - DNA, 20 bp, Artificial sequence
  Synthetic oligonucleotide
tcctcagttatccttgtgcc

SEQ ID NO: 47 - DNA, 20 bp, Artificial sequence
  Synthetic oligonucleotide
ttcaacctagactcagaggg

SEQ ID NO: 48 - DNA, 20 bp, Artificial sequence
  Synthetic oligonucleotide
atacctcttcccaatgctga

SEQ ID NO: 49 - DNA, 20 bp, Artificial sequence
  Synthetic oligonucleotide
acccaaacttgaccagctcc

SEQ ID NO: 50 - DNA, 20 bp, Artificial sequence
  Synthetic oligonucleotide
tcttgtcatttagaggccca

SEQ ID NO: 51 - DNA, 20 bp, Artificial sequence
  Synthetic oligonucleotide
gttgaaagacctgatatttg

SEQ ID NO: 52 - DNA, 20 bp, Artificial sequence
  Synthetic oligonucleotide
tgccgggtagcagtgctcaa

SEQ ID NO: 53 - DNA, 20 bp, Artificial sequence
  Synthetic oligonucleotide
tacttgggaaaaatgtgccc

SEQ ID NO: 54 - DNA, 20 bp, Artificial sequence
  Synthetic oligonucleotide
gcaagaaatagtcagttacc

SEQ ID NO: 55 - DNA, 20 bp, Artificial sequence
  Synthetic oligonucleotide
gtgccgaggaaaagggatcg

SEQ ID NO: 56 - DNA, 20 bp, Artificial sequence
  Synthetic oligonucleotide
ggataatgctttgggtacct

SEQ ID NO: 57 - DNA, 20 bp, Artificial sequence
  Synthetic oligonucleotide
ccacctgtgctaatgtttgc

SEQ ID NO: 58 - DNA, 20 bp, Artificial sequence
  Synthetic oligonucleotide
atgtgttgtgctccacctag

SEQ ID NO: 59 - DNA, 20 bp, Artificial sequence
  Synthetic oligonucleotide
gttatggtggaataatatgc

SEQ ID NO: 60 - DNA, 20 bp, Artificial sequence
  Synthetic oligonucleotide
ctggtggccccaactctacc

SEQ ID NO: 61 - DNA, 20 bp, Artificial sequence
  Synthetic oligonucleotide
ggccccctgtgacaggcata

SEQ ID NO: 62 - DNA, 20 bp, Artificial sequence
  Synthetic oligonucleotide
aactcctggaacgggttggc

SEQ ID NO: 63 - DNA, 20 bp, Artificial sequence
  Synthetic oligonucleotide
gtgtcctgctggtccaaaaa

SEQ ID NO: 64 - DNA, 20 bp, Artificial sequence
  Synthetic oligonucleotide
gggcccatgctacctgagac

SEQ ID NO: 65 - DNA, 20 bp, Artificial sequence
  Synthetic oligonucleotide
gaccttgctcaagctgaacc

SEQ ID NO: 66 - DNA, 20 bp, Artificial sequence
  Synthetic oligonucleotide
ggctctagtcaggactgtta

SEQ ID NO: 67 - DNA, 20 bp, Artificial sequence
  Synthetic oligonucleotide
gacaagggtatcttggtcct

SEQ ID NO: 68 - DNA, 20 bp, Artificial sequence
  Synthetic oligonucleotide
gcagtccaggtatcaaggcc

SEQ ID NO: 69 - DNA, 20 bp, Artificial sequence
  Synthetic oligonucleotide
taccccctctggtctgtgta

SEQ ID NO: 70 - DNA, 20 bp, Artificial sequence
  Synthetic oligonucleotide
gccatccacctgtagtagga

SEQ ID NO: 71 - DNA, 20 bp, Artificial sequence
  Synthetic oligonucleotide
gggcaacctacctgaacaag

SEQ ID NO: 72 - DNA, 20 bp, Artificial sequence
  Synthetic oligonucleotide
tgatggcccttttacctgac

SEQ ID NO: 73 - DNA, 20 bp, Artificial sequence
  Synthetic oligonucleotide
ggtttagccaaggccagtgc

SEQ ID NO: 74 - DNA, 20 bp, Artificial sequence
  Synthetic oligonucleotide
gcctggagttactcatgggc

SEQ ID NO: 75 - DNA, 20 bp, Artificial sequence
  Synthetic oligonucleotide
ggaccggaagtgcctttcgg

SEQ ID NO: 76 - DNA, 20 bp, Artificial sequence
  Synthetic oligonucleotide
gctggtcgcagcttgctccc

SEQ ID NO: 77 - DNA, 20 bp, Artificial sequence
  Synthetic oligonucleotide
gtgccacacttttcgacttc

SEQ ID NO: 78 - DNA, 20 bp, Artificial sequence
  Synthetic oligonucleotide
gagcgagcacgatggtaagg

SEQ ID NO: 79 - DNA, 20 bp, Artificial sequence
  Synthetic oligonucleotide
ggtaaacagtatcttcatcc

SEQ ID NO: 80 - DNA, 20 bp, Artificial sequence
  Synthetic oligonucleotide
tcagtcttattggaggtccc

SEQ ID NO: 81 - DNA, 20 bp, Artificial sequence
  Synthetic oligonucleotide
tccagcggctctaaaacaca

SEQ ID NO: 82 - DNA, 20 bp, Artificial sequence
  Synthetic oligonucleotide
gtgactaccctcaaaaggag

SEQ ID NO: 83 - DNA, 20 bp, Artificial sequence
  Synthetic oligonucleotide
ggctcggaatctctggctgc

SEQ ID NO: 84 - DNA, 20 bp, Artificial sequence
  Synthetic oligonucleotide
gctcaggagacattgaccat

SEQ ID NO: 85 - DNA, 20 bp, Artificial sequence
  Synthetic oligonucleotide
ggctctgatacatgtggcta

SEQ ID NO: 86 - DNA, 20 bp, Artificial sequence
  Synthetic oligonucleotide
ccatagcctcaagtcgatcc

SEQ ID NO: 87 - DNA, 20 bp, Artificial sequence
  Synthetic oligonucleotide
attttgattttgtggaacgc

SEQ ID NO: 88 - DNA, 20 bp, Artificial sequence
  Synthetic oligonucleotide
tcctcttagttcgagactcc

SEQ ID NO: 89 - DNA, 20 bp, Artificial sequence
  Synthetic oligonucleotide
ccctttcagaggccggttgt

SEQ ID NO: 90 - DNA, 20 bp, Artificial sequence
  Synthetic oligonucleotide
gcttggaggctgtccctcta

SEQ ID NO: 91 - DNA, 20 bp, Artificial sequence
  Synthetic oligonucleotide
gagatcttggcaacttgtcg

SEQ ID NO: 92 - DNA, 20 bp, Artificial sequence
  Synthetic oligonucleotide
gctgtgagaagggcccaact

SEQ ID NO: 93 - DNA, 20 bp, Artificial sequence
  Synthetic oligonucleotide
gggatctctgcccagtcaag

SEQ ID NO: 94 - DNA, 20 bp, Artificial sequence
  Synthetic oligonucleotide
ggcagctccgaaccctatgg

SEQ ID NO: 95 - DNA, 20 bp, Artificial sequence
  Synthetic oligonucleotide
aggctcattactctcagggt

SEQ ID NO: 96 - DNA, 20 bp, Artificial sequence
  Synthetic oligonucleotide
ccaggtgactcctatatatg

SEQ ID NO: 97 - DNA, 20 bp, Artificial sequence
  Synthetic oligonucleotide
tgccatctgcagctccgact

SEQ ID NO: 98 - DNA, 20 bp, Artificial sequence
  Synthetic oligonucleotide
tatacagcttgacaacctct

SEQ ID NO: 99 - DNA, 20 bp, Artificial sequence
  Synthetic oligonucleotide
gctctcctagatcagttgtt

SEQ ID NO: 100 - DNA, 20 bp, Artificial sequence
  Synthetic oligonucleotide
gcctccaagccctatgatgc

SEQ ID NO: 101 - DNA, 20 bp, Artificial sequence
  Synthetic oligonucleotide
tgggttagcagatgtcttcc

SEQ ID NO: 102 - DNA, 20 bp, Artificial sequence
  Synthetic oligonucleotide
gatgtcttaactcccctgtc

SEQ ID NO: 103 - DNA, 20 bp, Artificial sequence
  Synthetic oligonucleotide
ggtggtcaatattgacctgt

SEQ ID NO: 104 - DNA, 20 bp, Artificial sequence
  Synthetic oligonucleotide
taaccatgggatctagaagc

SEQ ID NO: 105 - DNA, 20 bp, Artificial sequence
  Synthetic oligonucleotide
ttggatggcaggtattgcat

SEQ ID NO: 106 - DNA, 20 bp, Artificial sequence
  Synthetic oligonucleotide
gtgcaccatgaacttctttg

SEQ ID NO: 107 - DNA, 20 bp, Artificial sequence
  Synthetic oligonucleotide
ctcttcactttctcggaagg

SEQ ID NO: 108 - DNA, 20 bp, Artificial sequence
  Synthetic oligonucleotide
caacactgatggccctttga

SEQ ID NO: 109 - DNA, 20 bp, Artificial sequence
  Synthetic oligonucleotide
gtgcatactggtctccacac

SEQ ID NO: 110 - DNA, 20 bp, Artificial sequence
  Synthetic oligonucleotide
tgtgtatcctaacccaagga

SEQ ID NO: 111 - DNA, 20 bp, Artificial sequence
  Synthetic oligonucleotide
cgattcattagtggcttcag

SEQ ID NO: 112 - DNA, 20 bp, Artificial sequence
  Synthetic oligonucleotide
ctccagatggaatttgtact

SEQ ID NO: 113 - DNA, 20 bp, Artificial sequence
  Synthetic oligonucleotide
gacactagcacctgtgcttg

SEQ ID NO: 114 - DNA, 20 bp, Artificial sequence
  Synthetic oligonucleotide
acctgtaattaggcccaggt

SEQ ID NO: 115 - DNA, 20 bp, Artificial sequence
  Synthetic oligonucleotide
catctgatatacccccaggc

SEQ ID NO: 116 - DNA, 20 bp, Artificial sequence
  Synthetic oligonucleotide
gccacacatcttaagtggga

SEQ ID NO: 117 - DNA, 20 bp, Artificial sequence
  Synthetic oligonucleotide
gcagtccctctacccatgca

SEQ ID NO: 118 - DNA, 20 bp, Artificial sequence
  Synthetic oligonucleotide
taacagccacccctgtcagg

SEQ ID NO: 119 - DNA, 20 bp, Artificial sequence
  Synthetic oligonucleotide
tctggactactttgaaccgg

SEQ ID NO: 120 - DNA, 20 bp, Artificial sequence
  Synthetic oligonucleotide
ggactataagtttcttggtg

SEQ ID NO: 121 - DNA, 20 bp, Artificial sequence
  Synthetic oligonucleotide
gcaatcatgggtttctacca

SEQ ID NO: 122 - DNA, 20 bp, Artificial sequence
  Synthetic oligonucleotide
ggcatataaccaagcatgag

SEQ ID NO: 123 - DNA, 20 bp, Artificial sequence
  Synthetic oligonucleotide
gttgggcccatccgtgtgtc

SEQ ID NO: 124 - DNA, 20 bp, Artificial sequence
  Synthetic oligonucleotide
atttacatttataccgccaa

SEQ ID NO: 125 - DNA, 20 bp, Artificial sequence
  Synthetic oligonucleotide
gatgggaaatgtgtgtagcc

SEQ ID NO: 126 - DNA, 20 bp, Artificial sequence
  Synthetic oligonucleotide
gtcaagaccttgggacatca

SEQ ID NO: 127 - DNA, 20 bp, Artificial sequence
  Synthetic oligonucleotide
ggaccaatccaggaaaggtt

SEQ ID NO: 128 - DNA, 20 bp, Artificial sequence
  Synthetic oligonucleotide
aggatggtgtataagcccta

SEQ ID NO: 129 - DNA, 20 bp, Artificial sequence
  Synthetic oligonucleotide
ggaactccacatttctaagc

SEQ ID NO: 130 - DNA, 20 bp, Artificial sequence
  Synthetic oligonucleotide
ggaggttcagtcttgaggca

SEQ ID NO: 131 - DNA, 20 bp, Artificial sequence
  Synthetic oligonucleotide
ggttgtgctgaaatatggtc

SEQ ID NO: 132 - DNA, 20 bp, Artificial sequence
  Synthetic oligonucleotide
gggtcacctttgttgcccat

SEQ ID NO: 133 - DNA, 20 bp, Artificial sequence
  Synthetic oligonucleotide
tgtccagttcggttcccatc

SEQ ID NO: 134 - DNA, 20 bp, Artificial sequence
  Synthetic oligonucleotide
cctggaagtacattgggacc

SEQ ID NO: 135 - DNA, 20 bp, Artificial sequence
  Synthetic oligonucleotide
ttgctctatactgtgatgac

SEQ ID NO: 136 - DNA, 20 bp, Artificial sequence
  Synthetic oligonucleotide
ctcctctgatcatgtacccc

SEQ ID NO: 137 - DNA, 20 bp, Artificial sequence
  Synthetic oligonucleotide
cacactttgcagttacctat

SEQ ID NO: 138 - DNA, 20 bp, Artificial sequence
  Synthetic oligonucleotide
ggcaacctgtcaaagcctta

SEQ ID NO: 139 - DNA, 20 bp, Artificial sequence
  Synthetic oligonucleotide
ccctagtttgccagggctcc

SEQ ID NO: 140 - DNA, 20 bp, Artificial sequence
  Synthetic oligonucleotide
gggaccctcctgttgtaagt

SEQ ID NO: 141 - DNA, 20 bp, Artificial sequence
  Synthetic oligonucleotide
cagtgctatcatgatcaggt

SEQ ID NO: 142 - DNA, 20 bp, Artificial sequence
  Synthetic oligonucleotide
cccagagatttggtatgggc

SEQ ID NO: 143 - DNA, 20 bp, Artificial sequence
  Synthetic oligonucleotide
gctccttagctaatctctga

SEQ ID NO: 144 - DNA, 20 bp, Artificial sequence
  Synthetic oligonucleotide
gattaggaaggctgtttagc

SEQ ID NO: 145 - DNA, 20 bp, Artificial sequence
  Synthetic oligonucleotide
ggagatagcggatggaatac

SEQ ID NO: 146 - DNA, 20 bp, Artificial sequence
  Synthetic oligonucleotide
ttatcctccccctacaaacc

SEQ ID NO: 147 - DNA, 20 bp, Artificial sequence
  Synthetic oligonucleotide
cagatctgctatccgggtgt

SEQ ID NO: 148 - DNA, 20 bp, Artificial sequence
  Synthetic oligonucleotide
taacaccaggccgaaggtca

SEQ ID NO: 149 - DNA, 20 bp, Artificial sequence
  Synthetic oligonucleotide
ttgcagattgctggataggg

SEQ ID NO: 150 - DNA, 20 bp, Artificial sequence
  Synthetic oligonucleotide
aaggttcagactatgggagg

SEQ ID NO: 151 - DNA, 20 bp, Artificial sequence
  Synthetic oligonucleotide
tagtctcagagggaccctta

SEQ ID NO: 152 - DNA, 20 bp, Artificial sequence
  Synthetic oligonucleotide
ctcagtccctcacacgatgc

SEQ ID NO: 153 - DNA, 20 bp, Artificial sequence
  Synthetic oligonucleotide
gtcatcactctggtcaacat

SEQ ID NO: 154 - DNA, 20 bp, Artificial sequence
  Synthetic oligonucleotide
aaagagccactaggttcatc

SEQ ID NO: 155 - DNA, 20 bp, Artificial sequence
  Synthetic oligonucleotide
ttgataggccaagataccca

SEQ ID NO: 156 - DNA, 20 bp, Artificial sequence
  Synthetic oligonucleotide
gctgtctatgattagaaccc

SEQ ID NO: 157 - DNA, 20 bp, Artificial sequence
  Synthetic oligonucleotide
ctcaaaaggtgcagggtccc

SEQ ID NO: 158 - DNA, 20 bp, Artificial sequence
  Synthetic oligonucleotide
acttgtcgattgcttggagg

SEQ ID NO: 159 - DNA, 20 bp, Artificial sequence
  Synthetic oligonucleotide
ggtactgattatgatgggac

SEQ ID NO: 160 - DNA, 20 bp, Artificial sequence
  Synthetic oligonucleotide
ggtcccctcctgaacccatg

SEQ ID NO: 161 - DNA, 20 bp, Artificial sequence
  Synthetic oligonucleotide
gcatcaggatctgttggcca

SEQ ID NO: 162 - DNA, 20 bp, Artificial sequence
  Synthetic oligonucleotide
aggaactcaaccttcgcacg

SEQ ID NO: 163 - DNA, 20 bp, Artificial sequence
  Synthetic oligonucleotide
ggttgcaacacagtgaggct

SEQ ID NO: 164 - DNA, 20 bp, Artificial sequence
  Synthetic oligonucleotide
gtaaaagtaactcctggcac

SEQ ID NO: 165 - DNA, 20 bp, Artificial sequence
  Synthetic oligonucleotide
gaatgttcctctatagcagt

SEQ ID NO: 166 - DNA, 20 bp, Artificial sequence
  Synthetic oligonucleotide
gcacctcctaaaagctgtta

SEQ ID NO: 167 - DNA, 20 bp, Artificial sequence
  Synthetic oligonucleotide
ggtgacacaacatatcgccc

SEQ ID NO: 168 - DNA, 20 bp, Artificial sequence
  Synthetic oligonucleotide
cctatgatggacagctgcac

SEQ ID NO: 169 - DNA, 20 bp, Artificial sequence
  Synthetic oligonucleotide
agtacgggagaattttgcca

SEQ ID NO: 170 - DNA, 20 bp, Artificial sequence
  Synthetic oligonucleotide
ttaactactgacagatatcc

SEQ ID NO: 171 - DNA, 20 bp, Artificial sequence
  Synthetic oligonucleotide
cctgagtcaaggagtttagc

SEQ ID NO: 172 - DNA, 20 bp, Artificial sequence
  Synthetic oligonucleotide
gcagcaagagccgggaagta

SEQ ID NO: 173 - DNA, 20 bp, Artificial sequence
  Synthetic oligonucleotide
tatggctatagtctaacatc

SEQ ID NO: 174 - DNA, 20 bp, Artificial sequence
  Synthetic oligonucleotide
gttgctcataaccaatcccc

SEQ ID NO: 175 - DNA, 20 bp, Artificial sequence
  Synthetic oligonucleotide
acttctaggtgatgaatctg

SEQ ID NO: 176 - DNA, 20 bp, Artificial sequence
  Synthetic oligonucleotide
acatatgaggcataccacaa

SEQ ID NO: 177 - DNA, 20 bp, Artificial sequence
  Synthetic oligonucleotide
gtgtgacaaagccttctatc

SEQ ID NO: 178 - DNA, 20 bp, Artificial sequence
  Synthetic oligonucleotide
gctatcagggtgatatctac

SEQ ID NO: 179 - DNA, 20 bp, Artificial sequence
  Synthetic oligonucleotide
gtgttggtagtagaatgaag

SEQ ID NO: 180 - DNA, 20 bp, Artificial sequence
  Synthetic oligonucleotide
ggtagtagtcatgggcagct

SEQ ID NO: 181 - DNA, 20 bp, Artificial sequence
  Synthetic oligonucleotide
cacgctggcccctcccgctg

SEQ ID NO: 182 - DNA, 20 bp, Artificial sequence
  Synthetic oligonucleotide
ttcacggtagttatactcta

SEQ ID NO: 183 - DNA, 20 bp, Artificial sequence
  Synthetic oligonucleotide
gttatccttgtgccacttgg

SEQ ID NO: 184 - DNA, 20 bp, Artificial sequence
  Synthetic oligonucleotide
gctatagtagaaccttgaag

SEQ ID NO: 185 - DNA, 20 bp, Artificial sequence
  Synthetic oligonucleotide
gtcgggctgtcacttagccc

SEQ ID NO: 186 - DNA, 20 bp, Artificial sequence
  Synthetic oligonucleotide
gtgtccttggacatttaccc

SEQ ID NO: 187 - DNA, 20 bp, Artificial sequence
  Synthetic oligonucleotide
cgagagagactcctagagct

SEQ ID NO: 188 - DNA, 20 bp, Artificial sequence
  Synthetic oligonucleotide
gacctgatatttgcctccat

SEQ ID NO: 189 - DNA, 20 bp, Artificial sequence
  Synthetic oligonucleotide
tagctcagcaggattcccct

SEQ ID NO: 190 - DNA, 20 bp, Artificial sequence
  Synthetic oligonucleotide
gatttggtataatttagtag

SEQ ID NO: 191 - DNA, 20 bp, Artificial sequence
  Synthetic oligonucleotide
aagtaaccccttagctgtgt

SEQ ID NO: 192 - DNA, 20 bp, Artificial sequence
  Synthetic oligonucleotide
ctaacatggcactgcatcca

SEQ ID NO: 193 - DNA, 20 bp, Artificial sequence
  Synthetic oligonucleotide
gcatgactaaagtgtaatca

SEQ ID NO: 194 - DNA, 20 bp, Artificial sequence
  Synthetic oligonucleotide
tacagcctgctcatggtggg

SEQ ID NO: 195 - DNA, 20 bp, Artificial sequence
  Synthetic oligonucleotide
ctccacctagtcctgtgccg

SEQ ID NO: 196 - DNA, 20 bp, Artificial sequence
  Synthetic oligonucleotide
gttctcaagcagggagaacc

SEQ ID NO: 197 - DNA, 20 bp, Artificial sequence
  Synthetic oligonucleotide
gccccaagtggagccagtgt

SEQ ID NO: 198 - DNA, 20 bp, Artificial sequence
  Synthetic oligonucleotide
gggcatcccattagacttcc

SEQ ID NO: 199 - DNA, 20 bp, Artificial sequence
  Synthetic oligonucleotide
ggcccgagctctgctcttat

SEQ ID NO: 200 - DNA, 20 bp, Artificial sequence
  Synthetic oligonucleotide
gctctggccacctatcatct

SEQ ID NO: 201 - DNA, 20 bp, Artificial sequence
  Synthetic oligonucleotide
gtatctgcacagctgagggt

SEQ ID NO: 202 - DNA, 20 bp, Artificial sequence
  Synthetic oligonucleotide
ctaatgacatatcactgggc

SEQ ID NO: 203 - DNA, 20 bp, Artificial sequence
  Synthetic oligonucleotide
gaatccccattgtcttggtg

SEQ ID NO: 204 - DNA, 20 bp, Artificial sequence
  Synthetic oligonucleotide
atctttagccacgactgtat

SEQ ID NO: 205 - DNA, 20 bp, Artificial sequence
  Synthetic oligonucleotide
acagggccttatctagagat

SEQ ID NO: 206 - DNA, 20 bp, Artificial sequence
  Synthetic oligonucleotide
tagctggagacccccatagc

SEQ ID NO: 207 - DNA, 20 bp, Artificial sequence
  Synthetic oligonucleotide
atacaaccccaggctgtcat

SEQ ID NO: 208 - DNA, 20 bp, Artificial sequence
  Synthetic oligonucleotide
tgccatgatggcatgtagga

SEQ ID NO: 209 - DNA, 20 bp, Artificial sequence
  Synthetic oligonucleotide
ggttcccgggataccatccc

SEQ ID NO: 210 - DNA, 20 bp, Artificial sequence
  Synthetic oligonucleotide
cctctcggaccggaagtgcc

SEQ ID NO: 211 - DNA, 20 bp, Artificial sequence
  Synthetic oligonucleotide
actccaggctggtcgcagct

SEQ ID NO: 212 - DNA, 20 bp, Artificial sequence
  Synthetic oligonucleotide
cccgaggagatgacttctgc

SEQ ID NO: 213 - DNA, 20 bp, Artificial sequence
  Synthetic oligonucleotide
ggtccattcattgtgccaca

SEQ ID NO: 214 - DNA, 20 bp, Artificial sequence
  Synthetic oligonucleotide
caccccagcctccgtatgtg

SEQ ID NO: 215 - DNA, 20 bp, Artificial sequence
  Synthetic oligonucleotide
gctaaactttccagcggctc

SEQ ID NO: 216 - DNA, 20 bp, Artificial sequence
  Synthetic oligonucleotide
ggaacagtgactaccctcaa

SEQ ID NO: 217 - DNA, 20 bp, Artificial sequence
  Synthetic oligonucleotide
atagcaatggctcggaatct

SEQ ID NO: 218 - DNA, 20 bp, Artificial sequence
  Synthetic oligonucleotide
cgatgcaaatgctcaggaga

SEQ ID NO: 219 - DNA, 20 bp, Artificial sequence
  Synthetic oligonucleotide
gagtcagaactcctagatcc

SEQ ID NO: 220 - DNA, 20 bp, Artificial sequence
  Synthetic oligonucleotide
gacccaggccttaaataagt

SEQ ID NO: 221 - DNA, 20 bp, Artificial sequence
  Synthetic oligonucleotide
tgagacacttatatgtctcc

SEQ ID NO: 222 - DNA, 20 bp, Artificial sequence
  Synthetic oligonucleotide
gggccaggaccatgaaactt

SEQ ID NO: 223 - DNA, 20 bp, Artificial sequence
  Synthetic oligonucleotide
gggtcccctttcagaggccg

SEQ ID NO: 224 - DNA, 20 bp, Artificial sequence
  Synthetic oligonucleotide
cgattgcttggaggctgtcc

SEQ ID NO: 225 - DNA, 20 bp, Artificial sequence
  Synthetic oligonucleotide
cttagaaacatgtggttccc

SEQ ID NO: 226 - DNA, 20 bp, Artificial sequence
  Synthetic oligonucleotide
agtatgctgtgagaagggcc

SEQ ID NO: 227 - DNA, 20 bp, Artificial sequence
  Synthetic oligonucleotide
tggccaatgaggcttttccc

SEQ ID NO: 228 - DNA, 20 bp, Artificial sequence
  Synthetic oligonucleotide
gctcccaggcagctccgaac

SEQ ID NO: 229 - DNA, 20 bp, Artificial sequence
  Synthetic oligonucleotide
tcaccatactatcatcaggt

SEQ ID NO: 230 - DNA, 20 bp, Artificial sequence
  Synthetic oligonucleotide
ggaagttcatactgtgtcag

SEQ ID NO: 231 - DNA, 20 bp, Artificial sequence
  Synthetic oligonucleotide
tctgtactatacagcttgac

SEQ ID NO: 232 - DNA, 20 bp, Artificial sequence
  Synthetic oligonucleotide
agctctcctagatcagttgt

SEQ ID NO: 233 - DNA, 20 bp, Artificial sequence
  Synthetic oligonucleotide
ggttcctagccaacagactc

SEQ ID NO: 234 - DNA, 20 bp, Artificial sequence
  Synthetic oligonucleotide
tgataggctatcattaacga

SEQ ID NO: 235 - DNA, 20 bp, Artificial sequence
  Synthetic oligonucleotide
cctcaatccctaagagacct

SEQ ID NO: 236 - DNA, 20 bp, Artificial sequence
  Synthetic oligonucleotide
tcagtaaaggccgcctgaca

SEQ ID NO: 237 - DNA, 20 bp, Artificial sequence
  Synthetic oligonucleotide
gtgtaatctgtatgggagaa

SEQ ID NO: 238 - DNA, 20 bp, Artificial sequence
  Synthetic oligonucleotide
tggcatcaaccatggttccc

SEQ ID NO: 239 - DNA, 20 bp, Artificial sequence
  Synthetic oligonucleotide
gtttgactggagttgcctgc

SEQ ID NO: 240 - DNA, 20 bp, Artificial sequence
  Synthetic oligonucleotide
tgactctatgatctatgtgc

SEQ ID NO: 241 - DNA, 20 bp, Artificial sequence
  Synthetic oligonucleotide
ttctagccagcctcaagcat

SEQ ID NO: 242 - DNA, 20 bp, Artificial sequence
  Synthetic oligonucleotide
ggcctatatggacccccaga

SEQ ID NO: 243 - DNA, 20 bp, Artificial sequence
  Synthetic oligonucleotide
ggacctgacatacgggctga

SEQ ID NO: 244 - DNA, 20 bp, Artificial sequence
  Synthetic oligonucleotide
caacctacttaacctgtctc

SEQ ID NO: 245 - DNA, 20 bp, Artificial sequence
  Synthetic oligonucleotide
gtggagatagaacgattcat

SEQ ID NO: 246 - DNA, 20 bp, Artificial sequence
  Synthetic oligonucleotide
gtagtcctctatagaaggca

SEQ ID NO: 247 - DNA, 20 bp, Artificial sequence
  Synthetic oligonucleotide
ccagggtattctggaatgat

SEQ ID NO: 248 - DNA, 20 bp, Artificial sequence
  Synthetic oligonucleotide
acctggcatgggtgctaacc

SEQ ID NO: 249 - DNA, 20 bp, Artificial sequence
  Synthetic oligonucleotide
gggtcatctgatataccccc

SEQ ID NO: 250 - DNA, 20 bp, Artificial sequence
  Synthetic oligonucleotide
ggagaggctatgcatggtaa

SEQ ID NO: 251 - DNA, 20 bp, Artificial sequence
  Synthetic oligonucleotide
tcgcacagaacacctcagag

SEQ ID NO: 252 - DNA, 20 bp, Artificial sequence
  Synthetic oligonucleotide
ggtgcacctctgcatgctgt

SEQ ID NO: 253 - DNA, 20 bp, Artificial sequence
  Synthetic oligonucleotide
ccctccagaaccccacttga

SEQ ID NO: 254 - DNA, 20 bp, Artificial sequence
  Synthetic oligonucleotide
gcctgggcagaagtaagccg

SEQ ID NO: 255 - DNA, 20 bp, Artificial sequence
  Synthetic oligonucleotide
gttatgcagtatctctctca

SEQ ID NO: 256 - DNA, 20 bp, Artificial sequence
  Synthetic oligonucleotide
agggcatataaccaagcatg

SEQ ID NO: 257 - DNA, 20 bp, Artificial sequence
  Synthetic oligonucleotide
ggttgggcccatccgtgtgt

SEQ ID NO: 258 - DNA, 20 bp, Artificial sequence
  Synthetic oligonucleotide
ggagagcataagccctagtg

SEQ ID NO: 259 - DNA, 20 bp, Artificial sequence
  Synthetic oligonucleotide
ggcaggtattaagttaccac

SEQ ID NO: 260 - DNA, 20 bp, Artificial sequence
  Synthetic oligonucleotide
ctgatgatgtggagggacca

SEQ ID NO: 261 - DNA, 20 bp, Artificial sequence
  Synthetic oligonucleotide
gggtactgttgctggcttgg

SEQ ID NO: 262 - DNA, 20 bp, Artificial sequence
  Synthetic oligonucleotide
gggccacaagtagcattcag

SEQ ID NO: 263 - DNA, 20 bp, Artificial sequence
  Synthetic oligonucleotide
gtgcccattgtcttctactc

SEQ ID NO: 264 - DNA, 20 bp, Artificial sequence
  Synthetic oligonucleotide
tggactgccagccctgattc

SEQ ID NO: 265 - DNA, 20 bp, Artificial sequence
  Synthetic oligonucleotide
gactcccaagggaggagacc

SEQ ID NO: 266 - DNA, 20 bp, Artificial sequence
  Synthetic oligonucleotide
cctagggcccagataggacc

SEQ ID NO: 267 - DNA, 20 bp, Artificial sequence
  Synthetic oligonucleotide
gggtgaacaagctttgcagg

SEQ ID NO: 268 - DNA, 20 bp, Artificial sequence
  Synthetic oligonucleotide
gtcctgtcagggcaagccat

SEQ ID NO: 269 - DNA, 20 bp, Artificial sequence
  Synthetic oligonucleotide
gcatatagagcctctgagac

SEQ ID NO: 270 - DNA, 20 bp, Artificial sequence
  Synthetic oligonucleotide
ggatccagagagtccctttg

SEQ ID NO: 271 - DNA, 20 bp, Artificial sequence
  Synthetic oligonucleotide
gacggtggctatgggcaggc

SEQ ID NO: 272 - DNA, 20 bp, Artificial sequence
  Synthetic oligonucleotide
cacctttaaatggagctaga

SEQ ID NO: 273 - DNA, 20 bp, Artificial sequence
  Synthetic oligonucleotide
cgtccttcctggcactgacc

SEQ ID NO: 274 - DNA, 20 bp, Artificial sequence
  Synthetic oligonucleotide
gccccctgtcttcaggtgtg

SEQ ID NO: 275 - DNA, 20 bp, Artificial sequence
  Synthetic oligonucleotide
accagacaccccaagttggg

SEQ ID NO: 276 - DNA, 20 bp, Artificial sequence
  Synthetic oligonucleotide
ggtggtcctaggagaggctt

SEQ ID NO: 277 - DNA, 20 bp, Artificial sequence
  Synthetic oligonucleotide
gttactcatgggcagccaga

SEQ ID NO: 278 - DNA, 20 bp, Artificial sequence
  Synthetic oligonucleotide
ggaagtgcctttcggacttc

SEQ ID NO: 279 - DNA, 20 bp, Artificial sequence
  Synthetic oligonucleotide
gtctcaagtggcaagtctgt

SEQ ID NO: 280 - DNA, 20 bp, Artificial sequence
  Synthetic oligonucleotide
tgccacacttttcgacttca

SEQ ID NO: 281 - DNA, 20 bp, Artificial sequence
  Synthetic oligonucleotide
cttattggaggtcccgtagg

SEQ ID NO: 282 - DNA, 20 bp, Artificial sequence
  Synthetic oligonucleotide
gacatgataacctagcacca

SEQ ID NO: 283 - DNA, 20 bp, Artificial sequence
  Synthetic oligonucleotide
gccagaggtctgtgcaatat

SEQ ID NO: 284 - DNA, 20 bp, Artificial sequence
  Synthetic oligonucleotide
gaccatattttatgtagcag

SEQ ID NO: 285 - DNA, 20 bp, Artificial sequence
  Synthetic oligonucleotide
ccatcagttactgtggataa

SEQ ID NO: 286 - DNA, 20 bp, Artificial sequence
  Synthetic oligonucleotide
cctcaagtcgatccacttgt

SEQ ID NO: 287 - DNA, 20 bp, Artificial sequence
  Synthetic oligonucleotide
acgctgtccagggctcacaa

SEQ ID NO: 288 - DNA, 20 bp, Artificial sequence
  Synthetic oligonucleotide
gttcgagactccagcccagc

SEQ ID NO: 289 - DNA, 20 bp, Artificial sequence
  Synthetic oligonucleotide
cagaggccggttgtctgtgc

SEQ ID NO: 290 - DNA, 20 bp, Artificial sequence
  Synthetic oligonucleotide
tctacctggaacacttagcc

SEQ ID NO: 291 - DNA, 20 bp, Artificial sequence
  Synthetic oligonucleotide
cttggcaacttgtcgattgc

SEQ ID NO: 292 - DNA, 20 bp, Artificial sequence
  Synthetic oligonucleotide
ggcccaactagggacaggtt

SEQ ID NO: 293 - DNA, 20 bp, Artificial sequence
  Synthetic oligonucleotide
gcaaggtatctgcttcttga

SEQ ID NO: 294 - DNA, 20 bp, Artificial sequence
  Synthetic oligonucleotide
cgaaccctatggaaagactc

SEQ ID NO: 295 - DNA, 20 bp, Artificial sequence
  Synthetic oligonucleotide
gggttagagcaagtatacca

SEQ ID NO: 296 - DNA, 20 bp, Artificial sequence
  Synthetic oligonucleotide
gagtgcagtgctattccttt

SEQ ID NO: 297 - DNA, 20 bp, Artificial sequence
  Synthetic oligonucleotide
gactacctactcagggtcct

SEQ ID NO: 298 - DNA, 20 bp, Artificial sequence
  Synthetic oligonucleotide
gttctcaatgtggtattccc

SEQ ID NO: 299 - DNA, 20 bp, Artificial sequence
  Synthetic oligonucleotide
ggcacacaggtgtagtgaat

SEQ ID NO: 300 - DNA, 20 bp, Artificial sequence
  Synthetic oligonucleotide
ggctgttaggtacaacgggc

SEQ ID NO: 301 - DNA, 20 bp, Artificial sequence
  Synthetic oligonucleotide
ggacttgcataggctggcag

SEQ ID NO: 302 - DNA, 20 bp, Artificial sequence
  Synthetic oligonucleotide
gtcagagtgtctataagcta

SEQ ID NO: 303 - DNA, 20 bp, Artificial sequence
  Synthetic oligonucleotide
atcaaacccgtcttctgcaa

SEQ ID NO: 304 - DNA, 20 bp, Artificial sequence
  Synthetic oligonucleotide
cagctcctgcaagtcagacg

SEQ ID NO: 305 - DNA, 20 bp, Artificial sequence
  Synthetic oligonucleotide
tctaagagtccaagcaactc

SEQ ID NO: 306 - DNA, 20 bp, Artificial sequence
  Synthetic oligonucleotide
tgtccagcatacttaggtct

SEQ ID NO: 307 - DNA, 20 bp, Artificial sequence
  Synthetic oligonucleotide
agtccaccgactcccagtga

SEQ ID NO: 308 - DNA, 20 bp, Artificial sequence
  Synthetic oligonucleotide
ggtttgggtgtgaatagtta

SEQ ID NO: 309 - DNA, 20 bp, Artificial sequence
  Synthetic oligonucleotide
aggtgcaaccagcactgtct

SEQ ID NO: 310 - DNA, 20 bp, Artificial sequence
  Synthetic oligonucleotide
tcccataactatctactgcc

SEQ ID NO: 311 - DNA, 20 bp, Artificial sequence
  Synthetic oligonucleotide
gagcaactccagcactaatt

SEQ ID NO: 312 - DNA, 20 bp, Artificial sequence
  Synthetic oligonucleotide
aggatcagatttgactccgt

SEQ ID NO: 313 - DNA, 20 bp, Artificial sequence
  Synthetic oligonucleotide
tggtcactaaagggataccc

SEQ ID NO: 314 - DNA, 20 bp, Artificial sequence
  Synthetic oligonucleotide
ctggtgttgtttcacggtag

SEQ ID NO: 315 - DNA, 20 bp, Artificial sequence
  Synthetic oligonucleotide
gcccagatataagcagtggc

SEQ ID NO: 316 - DNA, 20 bp, Artificial sequence
  Synthetic oligonucleotide
cccacactgcaagaagtggt

SEQ ID NO: 317 - DNA, 20 bp, Artificial sequence
  Synthetic oligonucleotide
ttagagaggtgccaaaggac

SEQ ID NO: 318 - DNA, 20 bp, Artificial sequence
  Synthetic oligonucleotide
gcacttttccacctccccga

SEQ ID NO: 319 - DNA, 20 bp, Artificial sequence
  Synthetic oligonucleotide
ggactactttgaaccgggtc

SEQ ID NO: 320 - DNA, 20 bp, Artificial sequence
  Synthetic oligonucleotide
gggtggtagcctctggttca

SEQ ID NO: 321 - DNA, 20 bp, Artificial sequence
  Synthetic oligonucleotide
atgccgggtagcagtgctca

SEQ ID NO: 322 - DNA, 20 bp, Artificial sequence
  Synthetic oligonucleotide
gtgtaacagggcatgtaacc

SEQ ID NO: 323 - DNA, 20 bp, Artificial sequence
  Synthetic oligonucleotide
ggctcataacatcccactct

SEQ ID NO: 324 - DNA, 20 bp, Artificial sequence
  Synthetic oligonucleotide
cgtgttgaccttggttggag

SEQ ID NO: 325 - DNA, 20 bp, Artificial sequence
  Synthetic oligonucleotide
gttttcaagtaagtgattcc

SEQ ID NO: 326 - DNA, 20 bp, Artificial sequence
  Synthetic oligonucleotide
gccattggccaaaggccatc

SEQ ID NO: 327 - DNA, 20 bp, Artificial sequence
  Synthetic oligonucleotide
cgagacactagtaccatgga

SEQ ID NO: 328 - DNA, 20 bp, Artificial sequence
  Synthetic oligonucleotide
gctggtgaattggagactct

SEQ ID NO: 329 - DNA, 20 bp, Artificial sequence
  Synthetic oligonucleotide
ttctgtcccataacctccgg

SEQ ID NO: 330 - DNA, 20 bp, Artificial sequence
  Synthetic oligonucleotide
tccctgcatagaggcagacc

SEQ ID NO: 331 - DNA, 20 bp, Artificial sequence
  Synthetic oligonucleotide
atgtcccatccctactgggc

SEQ ID NO: 332 - DNA, 20 bp, Artificial sequence
  Synthetic oligonucleotide
ggtgccttagacagccatcc

SEQ ID NO: 333 - DNA, 20 bp, Artificial sequence
  Synthetic oligonucleotide
tagccaaggctctgtttagc

SEQ ID NO: 334 - DNA, 20 bp, Artificial sequence
  Synthetic oligonucleotide
gggaggtgtcatgtccacct

SEQ ID NO: 335 - DNA, 20 bp, Artificial sequence
  Synthetic oligonucleotide
agtttgacagctgtatggac

SEQ ID NO: 336 - DNA, 20 bp, Artificial sequence
  Synthetic oligonucleotide
gtgctaatgaccctctctgg

SEQ ID NO: 337 - DNA, 20 bp, Artificial sequence
  Synthetic oligonucleotide
gccaaagttcactgagcacc

SEQ ID NO: 338 - DNA, 20 bp, Artificial sequence
  Synthetic oligonucleotide
accataggacctattttggg

SEQ ID NO: 339 - DNA, 20 bp, Artificial sequence
  Synthetic oligonucleotide
gccttcacttttgagtccac

SEQ ID NO: 340 - DNA, 20 bp, Artificial sequence
  Synthetic oligonucleotide
gggccagtatctccttactc

SEQ ID NO: 341 - DNA, 20 bp, Artificial sequence
  Synthetic oligonucleotide
agagccctttatgtttgggt

SEQ ID NO: 342 - DNA, 20 bp, Artificial sequence
  Synthetic oligonucleotide
ccagggtatgaactcttacc

SEQ ID NO: 343 - DNA, 20 bp, Artificial sequence
  Synthetic oligonucleotide
tctctgagtggttcccggga

SEQ ID NO: 344 - DNA, 20 bp, Artificial sequence
  Synthetic oligonucleotide
gctgtttagcctctcggacc

SEQ ID NO: 345 - DNA, 20 bp, Artificial sequence
  Synthetic oligonucleotide
gcggatggaatacagatgtg

SEQ ID NO: 346 - DNA, 20 bp, Artificial sequence
  Synthetic oligonucleotide
ggcagaatcccgaggagatg

SEQ ID NO: 347 - DNA, 20 bp, Artificial sequence
  Synthetic oligonucleotide
ccacaggtccattcattgtg

SEQ ID NO: 348 - DNA, 20 bp, Artificial sequence
  Synthetic oligonucleotide
ctaggtggacacattgggca

SEQ ID NO: 349 - DNA, 20 bp, Artificial sequence
  Synthetic oligonucleotide
atgggcaccccagcctccgt

SEQ ID NO: 350 - DNA, 20 bp, Artificial sequence
  Synthetic oligonucleotide
cctctagcagctcccgctca

SEQ ID NO: 351 - DNA, 20 bp, Artificial sequence
  Synthetic oligonucleotide
cctgtcaaacaggagtaact

SEQ ID NO: 352 - DNA, 20 bp, Artificial sequence
  Synthetic oligonucleotide
cagagggacccttagatagc

SEQ ID NO: 353 - DNA, 20 bp, Artificial sequence
  Synthetic oligonucleotide
tcacacgatgcaaatgctca

SEQ ID NO: 354 - DNA, 20 bp, Artificial sequence
  Synthetic oligonucleotide
ggtcaacatcttgtctggga

SEQ ID NO: 355 - DNA, 20 bp, Artificial sequence
  Synthetic oligonucleotide
gccactaggttcatctccta

SEQ ID NO: 356 - DNA, 20 bp, Artificial sequence
  Synthetic oligonucleotide
gccaagatacccagatttcc

SEQ ID NO: 357 - DNA, 20 bp, Artificial sequence
  Synthetic oligonucleotide
tatgattagaacccatgccc

SEQ ID NO: 358 - DNA, 20 bp, Artificial sequence
  Synthetic oligonucleotide
gtgcagggtcccctttcaga

SEQ ID NO: 359 - DNA, 20 bp, Artificial sequence
  Synthetic oligonucleotide
tgtcgattgcttggaggctg

SEQ ID NO: 360 - DNA, 20 bp, Artificial sequence
  Synthetic oligonucleotide
gattatgatgggacacttag

SEQ ID NO: 361 - DNA, 20 bp, Artificial sequence
  Synthetic oligonucleotide
acccatgttcttgggagcta

SEQ ID NO: 362 - DNA, 20 bp, Artificial sequence
  Synthetic oligonucleotide
atctgttggccaatgaggct

SEQ ID NO: 363 - DNA, 20 bp, Artificial sequence
  Synthetic oligonucleotide
ccttcgcacgcccatccttc

SEQ ID NO: 364 - DNA, 20 bp, Artificial sequence
  Synthetic oligonucleotide
agtacagtgttgttgctcct

SEQ ID NO: 365 - DNA, 20 bp, Artificial sequence
  Synthetic oligonucleotide
acctacttacctggatgccc

SEQ ID NO: 366 - DNA, 20 bp, Artificial sequence
  Synthetic oligonucleotide
tatttgactctcaaggagtc

SEQ ID NO: 367 - DNA, 20 bp, Artificial sequence
  Synthetic oligonucleotide
gggagtaagtcccagccctt

SEQ ID NO: 368 - DNA, 20 bp, Artificial sequence
  Synthetic oligonucleotide
gtgtgcctaaatccaggttt

SEQ ID NO: 369 - DNA, 20 bp, Artificial sequence
  Synthetic oligonucleotide
ggactcactcaagtattgtg

SEQ ID NO: 370 - DNA, 20 bp, Artificial sequence
  Synthetic oligonucleotide
ggaaaccaaccaacttggac

SEQ ID NO: 371 - DNA, 20 bp, Artificial sequence
  Synthetic oligonucleotide
tccagctcacataaggtgcc

SEQ ID NO: 372 - DNA, 20 bp, Artificial sequence
  Synthetic oligonucleotide
ccttctgccagtggtagatg

SEQ ID NO: 373 - DNA, 20 bp, Artificial sequence
  Synthetic oligonucleotide
gtgcacaaattcactcagcg

SEQ ID NO: 374 - DNA, 20 bp, Artificial sequence
  Synthetic oligonucleotide
tggtcactaagtgaccagac

SEQ ID NO: 375 - DNA, 20 bp, Artificial sequence
  Synthetic oligonucleotide
ggtcccccctctattttgct

SEQ ID NO: 376 - DNA, 20 bp, Artificial sequence
  Synthetic oligonucleotide
cactttaagaagacctctcc

SEQ ID NO: 377 - DNA, 20 bp, Artificial sequence
  Synthetic oligonucleotide
gctagatatacatagtcatc

SEQ ID NO: 378 - DNA, 20 bp, Artificial sequence
  Synthetic oligonucleotide
tgctggaaaacttatcttgc

SEQ ID NO: 379 - DNA, 20 bp, Artificial sequence
  Synthetic oligonucleotide
tcagggtgatatctactctc

SEQ ID NO: 380 - DNA, 20 bp, Artificial sequence
  Synthetic oligonucleotide
ggatgagttgtatttgagtt

SEQ ID NO: 381 - DNA, 20 bp, Artificial sequence
  Synthetic oligonucleotide
gtctagacctatcaaagtgg

SEQ ID NO: 382 - DNA, 20 bp, Artificial sequence
  Synthetic oligonucleotide
cccgctgtagtcctctatag

SEQ ID NO: 383 - DNA, 20 bp, Artificial sequence
  Synthetic oligonucleotide
ggtagttatactctaagcca

SEQ ID NO: 384 - DNA, 20 bp, Artificial sequence
  Synthetic oligonucleotide
gaacctctttcccggccctc

SEQ ID NO: 385 - DNA, 20 bp, Artificial sequence
  Synthetic oligonucleotide
acctaatggaaggcatggta

SEQ ID NO: 386 - DNA, 20 bp, Artificial sequence
  Synthetic oligonucleotide
tacccatgcaattctactcc

SEQ ID NO: 387 - DNA, 20 bp, Artificial sequence
  Synthetic oligonucleotide
caactctggaaccaagtccc

SEQ ID NO: 388 - DNA, 20 bp, Artificial sequence
  Synthetic oligonucleotide
tgtgacaacccacaacaacg

SEQ ID NO: 389 - DNA, 20 bp, Artificial sequence
  Synthetic oligonucleotide
tggatcatagctctgtccaa

SEQ ID NO: 390 - DNA, 20 bp, Artificial sequence
  Synthetic oligonucleotide
tttagtagggaggtctgcgg

SEQ ID NO: 391 - DNA, 20 bp, Artificial sequence
  Synthetic oligonucleotide
atgcagcaggttatccacac

SEQ ID NO: 392 - DNA, 20 bp, Artificial sequence
  Synthetic oligonucleotide
gctatctgcatactacctgc

SEQ ID NO: 393 - DNA, 20 bp, Artificial sequence
  Synthetic oligonucleotide
gaggctccctccgcaagagg

SEQ ID NO: 394 - DNA, 20 bp, Artificial sequence
  Synthetic oligonucleotide
gtagtaaaactgtggcaggt

SEQ ID NO: 395 - DNA, 20 bp, Artificial sequence
  Synthetic oligonucleotide
taggctgtcggcctctgagc

SEQ ID NO: 396 - DNA, 20 bp, Artificial sequence
  Synthetic oligonucleotide
catagggtactgttgctggc

SEQ ID NO: 397 - DNA, 20 bp, Artificial sequence
  Synthetic oligonucleotide
acatgcactatattgggcca

SEQ ID NO: 398 - DNA, 20 bp, Artificial sequence
  Synthetic oligonucleotide
aacctctttcttgtacaggg

SEQ ID NO: 399 - DNA, 20 bp, Artificial sequence
  Synthetic oligonucleotide
cgagctctgctcttatctca

SEQ ID NO: 400 - DNA, 20 bp, Artificial sequence
  Synthetic oligonucleotide
cctccatgggaattatcctc

SEQ ID NO: 401 - DNA, 20 bp, Artificial sequence
  Synthetic oligonucleotide
gatgcttgcagcagtatgcc

SEQ ID NO: 402 - DNA, 20 bp, Artificial sequence
  Synthetic oligonucleotide
agcagataggtccccttgag

SEQ ID NO: 403 - DNA, 20 bp, Artificial sequence
  Synthetic oligonucleotide
ggacaagtggagcatacttg

SEQ ID NO: 404 - DNA, 20 bp, Artificial sequence
  Synthetic oligonucleotide
gttggcatatagagcctctg

SEQ ID NO: 405 - DNA, 20 bp, Artificial sequence
  Synthetic oligonucleotide
gatgagtgagtgcctgacca

SEQ ID NO: 406 - DNA, 20 bp, Artificial sequence
  Synthetic oligonucleotide
ggctcacttatgaagtgtgc

SEQ ID NO: 407 - DNA, 20 bp, Artificial sequence
  Synthetic oligonucleotide
ggcccccatgaaccaggcag

SEQ ID NO: 408 - DNA, 20 bp, Artificial sequence
  Synthetic oligonucleotide
gccaataggatccctacctc

SEQ ID NO: 409 - DNA, 20 bp, Artificial sequence
  Synthetic oligonucleotide
ctcattatggctactctcca

SEQ ID NO: 410 - DNA, 20 bp, Artificial sequence
  Synthetic oligonucleotide
gatccaagtccctgcatagt

SEQ ID NO: 411 - DNA, 20 bp, Artificial sequence
  Synthetic oligonucleotide
ccttccctgaaggttcctcc